European Patent Specification EP 3 280 267 B1, published November 5, 2025. Title: Proteases for High Protein Fermented Milk Products. Applicant: DuPont Nutrition Biosciences ApS E,I. DU PONT DE NEMOURS AND COMPANY Eisele, Thomas Bejder, Hans Christian D'Argence Vargas, Enrique Guillermo. The sequence listing filed with the application follows.

SEQUENCE LISTING (23 sequences)

SEQ ID NO: 1 - protein, 270 aa, Artificial Sequence
  Example protease sequence
AQSVPWGISRVQAPAAHNRGLTGSGVKVAVLDTGISTHPDLNIRGGASFVPGEPSTQDGNGHGTHVAGTIAALDNSIGVLGVAPSAELYAVKVLGASGSGAISSIAQGLEWAGNNGMHVANLSLGSPSPSATLEQAVNSATSRGVLVVAASGNSGAGSISYFPARYANAMAVGATDQNNNRASFSQYGAGLDIVAPGVNVQSTYPGSTYASLNGTSMATPHVAGAAALVKQKNPSWSNVQIRNHLKNTATSLGSTNLYGSGLVNAEAATR

SEQ ID NO: 2 - protein, 274 aa, Artificial Sequence
  Example protease sequence
AQTVPYGIPLIKADKVQAQGFKGANVKVAVLDTGIQASHPDLNVVGGASFVAGEAYNTDGNGHGTHVAGTVAALDNTTGVLGVAPSVSLYAVKVLNSSGSGSYSGIVSGIEWATTNGMDVINMSLGGASGSTAMKQAVDNAYARGVVVVAAAGNSGSSGNTNTIGYPAKYDSVIAVGAVDSNSNRASFSSVGAELEVMAPGAGVYSTYPTNTYATLNGTSMASPHVAGAAALILSKHPNLSASQVRNRLSSTATYLGSSFYYGKGLINVEAAAQ

SEQ ID NO: 3 - protein, 521 aa, Bacillus amyloliquefaciens
MGLGKKLSVAVAASFMSLTISLPGVQAAENPQLKENLTNFVPKHSLVQSELPSVSDKAIKQYLKQNGKVFKGNPSERLKLIDQTTDDLGYKHFRYVPVVNGVPVKDSQVIIHVDKSNNVYAINGELNNDVSAKTANSKKLSANQALDHAYKAIGKSPEAVSNGTVANKNKAELKAAATKDGKYRLAYDVTIRYIEPEPANWEVTVDAETGKILKKQNKVEHAATTGTGTTLKGKTVSLNISSESGKYVLRDLSKPTGTQIITYDLQNREYNLPGTLVSSTTNQFTTSSQRAAVDAHYNLGKVYDYFYQKFNRNSYDNKGGKIVSSVHYGSRYNNAAWIGDQMIYGDGDGSFFSPLSGSMDVTAHEMTHGVTQETANLNYENQPGALNESFSDVFGYFNDTEDWDIGEDITVSQPALRSLSNPTKYGQPDNFKNYKNLPNTDAGDYGGVHTNSGIPNKAAYNTITKIGVNKAEQIYYRALTVYLTPSSTFKDAKAALIQSARDLYGSQDAASVEAAWNAVGL

SEQ ID NO: 4 - protein, 300 aa, Bacillus pumilus
AAATGSGTTLKGATVPLNISYEGGKYVLRDLSKPTGTQIITYDLQNRQSRLPGTLVSSTTKTFTSSSQRAAVDAHYNLGKVYDYFYSNFKRNSYDNKGSKIVSSVHYGTQYNNAAWTGDQMIYGDGDGSFFSPLSGSLDVTAHEMTHGVTQETANLIYENQPGALNESFSDVFGYFNDTEDWDIGEDITVSQPALRSLSNPTKYNQPDNYANYRNLPNTDEGDYGGVHTNSGIPNKAAYNTITKLGVSKSQQIYYRALTTYLTPSSTFKDAKAALIQSARDLYGSTDAAKVEAAWNAVGL

SEQ ID NO: 5 - protein, 520 aa, Bacillus amyloliquefaciens
MGLGKKLSVAVAASFMSLTISLPGVQAAENPQLKENLTNFVPKHSLVQSELPSVSDKAIKQYLKQNGKVFKGNPSERLKLIDQTTDDLGYKHFRYVPVVNGVPVKDSQVIIHVDKSNNVYAINGELNNDVSAKTANSKKLSANQALDHAYKAIGKSPEAVSNGTVANKNKAELKAAATKDGKYRLAYDVTIRYIEPEPANWEVTVDAETGKILKKQNKVEHAATTGTGTTLKGKTVSLNISSESGKYVLRDLSKPTGTQIITYDLQNREYNLPGTLVSSTTNQFTTSSQRAAVDAHYNLGKVYDYFYQKFNRNSYDNKGGKIVSSVHYGSRYNNAAWIGDQMIYGDGDGSFFSPLSGSMDVTAHEMTHGVTQETANLNYENQPGALNESFSDVFGYFNDTEDWDIGEDITSQPALRSLSNPTKYGQPDNFKNYKNLPNTDAGDYGGVHTNSGIPNKAAYNTITKIGVNKAEQIYYRALTVYLTPSSTFKDAKAALIQSARDLYGSQDAASVEAAWNAVGL

SEQ ID NO: 6 - protein, 547 aa, Bacillus thermoproteolyticus
MKMKMKLASFGLAAGLAAQVFLPYNALASTEHVTWNQQFQTPQFISGDLLKVNGTSPEELVYQYVEKNENKFKFHENAKDTLQLKEKKNDNLGFTFMRFQQTYKGIPVFGAVVTSHVKDGTLTALSGTLIPNLDTKGSLKSGKKLSEKQARDIAEKDLVANVTKEVPEYEQGKDTEFVVYVNGDEASLAYVVNLNFLTPEPGNWLYIIDAVDGKILNKFNQLDAAKPGDVKSITGTSTVGVGRGVLGDQKNINTTYSTYYYLQDNTRGGIFTYDAKYRTTLPGSLWADADNQFFASYDAPAVDAHYYAGVTYDYYKNVHNRLSYDGNNAAIRSSVHYSQGYNNAFWNGSQMVYGDGDGQTFIPLSGGIDVVAHELTHAVTDYTAGLIYQNESGAINEAMSDIFGTLVKFYANKNPDWEIGEDVYTPGISGDSLRSMSDPAKYGDPDHYSKRYTGTQDNGGVHINSGIINKAAYLISQGGTHYGVSVVGIGRDKLGKIFYRALTQYLTPTSNFSQLRAAAVQSATDLYGSTSQEVASVKQAFDAVGVK

SEQ ID NO: 7 - protein, 314 aa, Penicillium oxalicum
MVCHSLAPFVVLVTSLFFLQAKCSPVVFEQRGICATEDPDTSFLDALERVRTDETQLPDTGSEARNGPIEIETWFHIITSKAEQDQVSDDMIESQISILQDAYQDAGIQYRLQGVTRHVNDVWARNGDDTGMKSALRKGTYRTLNVYFQTDLQASPDQAGRASHRGASHSSDLSSSVLGFCTLPDPSVNATSPRADYIKDGCNVLASAMSGGTLDLYNRGGTAIHEIGHWNGLLHTFQGESCAEDNPGDYIADTPQQSVPTGGCPARKDSCPNLPGQDPIHDFMDYSSDVCYESFTPGQNERMRNMWASMRAGK

SEQ ID NO: 8 - DNA, 1023 bp, Penicillium oxalicum
atggtctgtcactctttagctccgttcgtggttcttgtcacatctctctttttcttgcaagcgaaatgcagccccgtggtgtttgaacagcgtggcatctgcgctaccgaagatccagatacgtccttcttggacgcactcgagcgtgtcagaacagatgagacccagctacctgacactgggtcagaggcccgcaacggccccatcgagattgagacctggttccatatcatcaccagcaaagcagagcaagaccaggtttctgatgacatgatcgagtcccaggtaagtcctacctccatcgctcctgttctcgacgacttcaatcgcatgtcatgaacgaatgctaagacactcgcctagatctccattctacaagatgcgtatcaggatgccggtattcaatatcgactgcaaggtgtcacccgccatgtgaacgatgtttgggctcgcaacggagatgacacaggcatgaagtcagcccttcgaaaagggacctatcggactctaaacgtttacttccaaaccgacctccaggcatcacccgaccaagccggtcgtgcaagccaccgcggagcttctcattcaagtgatctctcatccagcgtgctaggattctgcaccctccccgatccaagcgtgaatgccaccagtccccgtgccgactacattaaggatggctgcaacgttctcgctagcgcgatgtccggaggcacattggacctttacaaccgaggaggaaccgccatccacgagatcggacattggaatggccttttgcataccttccaaggggagtcctgtgccgaggataatccaggggactacattgccgacacgccccaacaatctgtcccaactggcggatgccctgctcgaaaggattcttgtcccaatttgccggggcaggaccccatccacgactttatggactactcatctgatgtctgttatgagagttttacacctggtcagaatgaacgtatgcgaaatatgtgggcatcgatgcgtgcagggaaatag

SEQ ID NO: 9 - protein, 318 aa, Aspergillus oryzae
MSHFPTLHILILVIANLQIQCFAFVSQSRGFCATGPPTESLKAEYRRLSALGSQSYNPVDSESRAAITPIVIDTWFHIITGEAGTELISDEMIADQLSYLQNAYWNATISYRLQGVTRSANDTWARNEDEMAMKTVLRRGSYRTLNVYFHTDLQASPNAGARAFDIVRRELGVSQQQPTSMLGFCTLPDPSINASSPPSTYIKDGCNVLAETMPGGSLAHYNRGGTAIHEIGHWNGLLHTFEGESCSSDNEGDFIADTPQQSKPTEGCPAQKDSCPELPGFDAIHNFMDYSSDECYDSFTPDQVSRMRSMWFAMRDGK

SEQ ID NO: 10 - DNA, 1908 bp, Bacillus amyloliquefaciens
gatcttaacatttttcccctatcatttttcccgtcttcatttgtcattttttccagaaaaaatcgcgtcattcgactcatgtctaatccaacacgtgtctctcggcttatcccctgacaccgcccgccgacagcccgcatgggacgattctatcaattcagccgcggagtctagttttatattgcagaatgcgagattgctggtttattataacaatataagttttcattattttcaaaaagggggatttattgtgggtttaggtaagaaattgtctgttgctgtcgccgcttcctttatgagtttaaccatcagtctgccgggtgttcaggccgctgagaatcctcagcttaaagaaaacctgacgaattttgtaccgaagcattctttggtgcaatcagaattgccttctgtcagtgacaaagctatcaagcaatacttgaaacaaaacggcaaagtctttaaaggcaatccttctgaaagattgaagctgattgaccaaacgaccgatgatctcggctacaagcacttccgttatgtgcctgtcgtaaacggtgtgcctgtgaaagactctcaagtcattattcacgtcgataaatccaacaacgtctatgcgattaacggtgaattaaacaacgatgtttccgccaaaacggcaaacagcaaaaaattatctgcaaatcaggcgctggatcatgcttataaagcgatcggcaaatcacctgaagccgtttctaacggaaccgttgcaaacaaaaacaaagccgagctgaaagcagcagccacaaaagacggcaaataccgcctcgcctatgatgtaaccatccgctacatcgaaccggaacctgcaaactgggaagtaaccgttgatgcggaaacaggaaaaatcctgaaaaagcaaaacaaagtggagcatgccgccacaaccggaacaggtacgactcttaaaggaaaaacggtctcattaaatatttcttctgaaagcggcaaatatgtgctgcgcgatctttctaaacctaccggaacacaaattattacgtacgatctgcaaaaccgcgagtataacctgccgggcacactcgtatccagcaccacaaaccagtttacaacttcttctcagcgcgctgccgttgatgcgcattacaacctcggcaaagtgtatgattatttctatcagaagtttaatcgcaacagctacgacaataaaggcggcaagatcgtatcctccgttcattacggcagcagatacaataacgcagcctggatcggcgaccaaatgatttacggtgacggcgacggttcattcttctcacctctttccggttcaatggacgtaaccgctcatgaaatgacacatggcgttacacaggaaacagccaacctgaactacgaaaatcagccgggcgctttaaacgaatccttctctgatgtattcgggtacttcaacgatactgaggactgggatatcggtgaagatattacggtcagccagccggctctccgcagcttatccaatccgacaaaatacggacagcctgataatttcaaaaattacaaaaaccttccgaacactgatgccggcgactacggcggcgtgcatacaaacagcggaatcccgaacaaagccgcttacaatacgattacaaaaatcggcgtgaacaaagcggagcagatttactatcgtgctctgacggtatacctcactccgtcatcaacttttaaagatgcaaaagccgctttgattcaatctgcgcgggacctttacggctctcaagatgctgcaagcgtagaagctgcctggaatgcagtcggattgtaaacaagaaaagagaccggaaatccggtctcttttttatatctaaaaacatttcacagtggcttcaccatgatcatatatgtcttttcccg

SEQ ID NO: 11 - protein, 521 aa, Bacillus subtilis
  misc_feature (338)..(338): Xaa can be any naturally occurring amino acid
MGLGKKLSVAVAASFMSLTISLPGVQAAENPQLKENLTNFVPKHSLVQSELPSVSDKAIKQYLKQNGKVFKGNPSERLKLIDHTTDDLGYKHFRYVPVVNGVPVKDSQVIIHVDKSNNVYAINGELNNDASAKTANSKKLSANQALDHAFKAIGKSPEAVSNGNVANKNKAELKAAATKDGKYRLAYDVTIRYIEPEPANWEVTVDAETGKVLKKQNKVEHAAATGTGTTLKGKTVSLNISSENGKYVMRDLSKPTGTQIITYDLQNRQYNLPGTLVSSTTNQFTTSSQRAAVDAHYNLGKVYDYFYQTFKRNSYDNRGGKIVSSVHYGSRYNNAAWXGDQMIYGDGDGSFFSPLSGSMDVTAHEMTHGVTQETANLNYENQPGALNESFSDVFGYFTDTEDWDIGEDITVSQPALRSLSNPTKYGQPDHYKNYQNLPNTDAGDYGGVHTNSGIPNKAAYNTITKIGVKKAEQIYYRALTVYLTPSSSFKDAKAALIQSARDLYGSQDAASVEAAWNAVGL

SEQ ID NO: 12 - protein, 354 aa, Elizabethkingia miricola
MRKLLIFSISAYLMAGIVSCKGVDSATPVTEDRLALNAVNAPADNTVNIKTFDKVKNAFGDGLSQSAEGTFTFPADVTTVKTIKMFIKNECPNKTCDEWDRYANVYVKNKTTGEWYEIGRFITPYWVGTEKLPRGLEIDVTDFKSLLSGNTELKIYTETWLAKGREYSVDFDIVYGTPDYKYSAVVPVIQYNKSSIDGVPYGKAHTLGLKKNIQLPTNTEKAYLRTTISGWGHAKPYDAGSRGCAEWCFRTHTIAINNANTFQHQLGALGCSANPINNQSPGNWAPDRAGWCPGMAVPTRIDVLNNSLTGSTFSYEYKFQSWTNNGTNGDAFYAISSFVIAKSNTPISAPVVTN

SEQ ID NO: 13 - protein, 567 aa, Elizabethkingia meningoseptica
MLFFLPLLKTNLMQKILLCSLITGAQMIFAQTYEITYQNSFEGKINPNQNHIISITNSDKTLLFNEKIKNKKADFPFEVNEINRKNNEVSQFAFLNNNEIVKTSDNTILAKQEFKPTSETGKILGYNVKKAVTSVNSNTIEVWYTNDLKVKGGPSILGQDLGLVLKTVRNGSSVVEATSVKKIKALDDQSLFNGKNITEKDALTYKDMIWKSRFITIPVFENETINFSDASKSDQVIQRFGNGTIILKKVKIPEIKQGNTIFVELKQKSNGDAYDRTGDVFIIPQERAISYYTGLTQGVKSLPVYQNGNGKSYQGVALTPDYLPFIELMRFFTPFGIGHFNEKIQLKGKNWHNNTPYRQDITELRPQLSGKEILIGAFIGNYDKGGHQISLELSIHPDQQKIVNNNFVLPVFNTTNVMEMAGQDYPTMFNSDKGVEVEFILTKDLKNAQLRYITTGHGGWGAGDEFVPKENSIYLDGKLAHAFTPWRTDCGSYRLFNPASGNFEDGLSSSDLSRSNWCPGTITNPVYINLGNLNAGKHTIQVKIPQGAPEGSSQSFWNVSGVLLGQE

SEQ ID NO: 14 - protein, 313 aa, Streptomyces plicatus
MFTPVRRRVRTAALALSAAAALVLGSTAASGASATPSPAPAPAPAPVKQGPTSVAYVEVNNNSMLNVGKYTLADGGGNAFDVAVIFAANINYDTGTKTAYLHFNENVQRVLDNAVTQIRPLQQQGIKVLLSVLGNHQGAGFANFPSQQAASAFAKQLSDAVAKYGLDGVDFDDEYAEYGNNGTAQPNDSSFVHLVTALRANMPDKIISLYNIGPAASRLSYGGVDVSDKFDYAWNPYYGTWQVPGIALPKAQLSPAAVEIGRTSRSTVADLARRTVDEGYGVYLTYNLDGGDRTADVSAFTRELYGSEAVRTP

SEQ ID NO: 15 - protein, 243 aa, Schistosoma japonicum
MIFYRLLGLIFILETIILISSNVYGLDNGLARTPPMGWMTWQRFRCQIDCKEYPNDCINENLIKRTADKLVLNGWRDLGYKYVIIDDCWPARKRDSKTNELVPDPDRFPNGMKNVGEYLHSKNLLFGIYLDYGTLTCEGYPGSMNYLELDARSIAEWKVDYVKMDGCYSLPNIQPEGYENFSRLLNTTGRPMVFSCSYPAYISWINNIKLIDWNRLKKNCNLWRVLGDIQDSLSSVVSIIKCL

SEQ ID NO: 16 - protein, 592 aa, Paenibacillus polymyxa
MKKVWFSLLGGAMLLGSVASGASAESSVSGPAQLTPTFHAEQWKAPSSVSGDDIVWSYLNRQKKSLLGVDSSSVREQFRIVDRTSDKSGVSHYRLKQYVNGIPVYGAEQTIHVGKSGEVTSYLGAVINEDQQEEATQGTTPKISASEAVYTAYKEAAARIEALPTSDDTISKDAEEPSSVSKDTYAEAANNDKTLSVDKDELSLDKASVLKDSKIEAVEAEKSSIAKIANLQPEVDPKAELYYYPKGDDLLLVYVTEVNVLEPAPLRTRYIIDANDGSIVFQYDIINEATGTGKGVLGDSKSFTTTASGSSYQLKDTTRGNGIVTYTASNRQSIPGTLLTDADNVWNDPAGVDAHAYAAKTYDYYKSKFGRNSIDGRGLQLRSTVHYGSRYNNAFWNGSQMTYGDGDGSTFIAFSGDPDVVGHELTHGVTEYTSNLEYYGESGALNEAFSDVIGNDIQRKNWLVGDDIYTPNIAGDALRSMSNPTLYDQPDHYSNLYKGSSDNGGVHTNSGIINKAYYLLAQGGTFHGVTVNGIGRDAAVQIYYSAFTNYLTSSSDFSNARAAVIQAAKDLYGANSAEATAAAKSFDAVGVN

SEQ ID NO: 17 - protein, 504 aa, Serratia liquefaciens
MSICLIENNQLMSGIEPMQSTKKAIEITESSLAAAGSGYNAVDDLLHYHERGNGIQVNGKDSFSTEQAGLFITRENQTWNGYKVFGQPVKLTFSFPDYKFSSTNVAGDTGLSKFSAEQQQQAKLSLQSWSDVANITFTEVGAGQKANITFGNYSQDRPGHYDYDTQAYAFLPNTIYQGQNLGGQTWYNVNQSNVKHPASEDYGRQTFTHEIGHALGLSHPGDYNAGEGNPTYRDASYAEDTREFSLMSYWSETNTGGDNGGHYAAAPLLDDISAIQHLYGANLTTRTGDTVYGFNSNTGRDFLSTTSNSQKVIFAAWDAGGNDTFDFSGYTANQRINLNEKSFSDVGGLKGNVSIAAGVTIENAIGGSGNDVIVGNAANNVLKGGAGNDVLFGGGGADELWGGAGKDTFVFSAVSDSAPGASDWIKDFQKGIDKIDLSFFNQGAQGGDQIHFVDHFSGAAGEALLSYNASNNVSDLALNIGGHQAPDFLVKIVGQVDVATDFIV

SEQ ID NO: 18 - protein, 369 aa, Aspergillus niger
MSARNNHTYTFIQPQILQHISTSPNASSKARRAATRTLTLANEIHQTRVSSSPYISLTSHAQAREIYDCRNKRGLPGLLVRTESSSAPTTQDDTVNHVYNSFGIFLHFLSSVLGRQSIDNDNLRLIGCLHYDKNLDNAFWNGQEIIFGDGDGVYFAGFPKSLDVVVHELMHGVTDHTAGLLYEGQSGALSESISDVFACVIEQWWRGQGVEEADWVVGRGVFVWPKGKKGAGAGAGEMGLRSLKAPGTAYDDPVLGRDGQPSHMKELVCTEEDNGGVHWNSGIPSHAFYLCAVEFGGRSWEKAAIVWYRALLDPRVEPNCSFQRFASVTVDIAEAMFGGEAGEVVKRAWVAVGVEVGMVLWTVKGDTGC

SEQ ID NO: 19 - protein, 375 aa, Aspergillus terreus
MAHLCAFVPQYVLEGIVEKGLAPEHIINRCQSTIDKTTQLRDTRGRHVQSIAAAQQQRISQGIIPPYILESIARNPATEQQREAARHTLALSTKHRTAAARGGKLLSEAEDPTNNANECYNGLGKSYDFYFNFFQRNSVDDNGFELDGFVHAGDLYNAYWDGYELVFGDGDGVIFDGFTDELDVIGHEFSHGVVEHTSPLPYAFQSGALNESLADAFGVMIKQWGEGTPKTVDQADWLVGEGIWAEGVNGRALRDMANPGTAYDDPRVGKDPQPAHWKDFKKLSASDDEGGVHINSGIPNRAFYLAATKIGGYAWEGAGAIWYRALASGKLRKDGKAKFKDFADLTIENAGEHVDKVREAWTLVGYPFAEERHEL

SEQ ID NO: 20 - protein, 319 aa, Aspergillus kawachii
MTLLLNLHALFTAIVFANLSTRCSALLSGRDFCSTPAPDESLRAEHRRLYDLQAQRGSTAEESREVVSMIEIETWFHIVSSNEASNAVSDDMITSQLSYLQKAYESATISYRLEGITRHINDSWARNDDELGMKNALRRGIYSTLNVYFQTDLQASSDDTSRGFPYNGNRRTDVSGQSSTTVLGFCTLPDPSVNSSSPRSSYIKDGCNVLADTMPGGSLAQYNQGGTAVHEVGHWNGLLHTFEGESCSPDNEGDYIDDTPEQSEPTSGCPAEKDSCPDLPGLDAIHNFMDYSSDDCYESFTPDQAERMRSMWSAMREGK

SEQ ID NO: 21 - protein, 318 aa, Aspergillus oryzae; identical to SEQ ID NO: 9

SEQ ID NO: 22 - protein, 311 aa, Penicillium roqueforti
MVCHSFFQLVIFITVFLQAWCSPFALQKRGACATEDPGANFLHEVRRLQSDEADLAISQARKAPIEIETWFHIISSKSESTQVTDNMINSQFSILQQSYADSGISYRLQGVTRNVNDKWASNADDTAMKTTLRKGSYRTLNVYFQTDLQASPEQAGRAFGHRGAVTNNDLASSVLGFCTLPDPSVNASSPASQYIKDGCNVLAKTMPGGSLDLYNRGGTAIHEIGHWNGLLHTFQGESCSVDNPGDHISDTPQQSTPTDGCPDQKDSCPDSPGLDAVHDFMDYSSDVCYERFTPGQGERMRSMWISMREGK

SEQ ID NO: 23 - protein, 5 aa, Artificial Sequence
  Sequence motif
  misc_feature (3)..(4): Xaa can be any naturally occurring amino acid
HEXXH